European Patent Application EP 4 567 426 A1, published June 11, 2025. Title: A Nanoparticle, a Suspension Comprising Nanoparticles, and Related Methods. Applicant: Helmholtz Zentrum München Deutsches Forschungszentrum für Gesundheit und Umwelt (GmbH). Application EP. The sequence listing filed with the application follows.

SEQUENCE LISTING (5 sequences)

SEQ ID NO: 1 - protein, 60 aa, unidentified
MKHHHHHHPMEPLSQETFSDLWKLLPENNVLSPLPSQAMDDLMLSPDDIEQWFTEDPGPD

SEQ ID NO: 2 - protein, 63 aa, unidentified
GAMEPPRSISPSALQDLLRTLKSPSSPQQQQQVLNILKSNPQLMAAFIKQRTAKYVANQPGMQ

SEQ ID NO: 3 - protein, 122 aa, unidentified
MKHHHHHHPMAMRELVEAECGGANPLMKLAGHFTQDKALRQEGLRPGPWPPGAPASEAASKPLGVASEDELVAEFLQDQNAPLVSRAPQTFKMDDLLAEMQQIEQSNFRQAPQRAPGVADLA

SEQ ID NO: 4 - protein, 131 aa, unidentified
MKHHHHHHPMADLALSENWAQEFLAAGDAVDVTQDYNETDWSQEFISEVTDPLSVSPARWAEEYLEQSEEKLWLGEPEGTATDRWYDEYHPEEDLQHTASDFVAKVDDPKLANSEFLKFVRQIGEGQVSLE

SEQ ID NO: 5 - protein, 70 aa, unidentified
GAMATPGSENVLPREPLIATAVKFLQNSRVRQSPLATRRAFLKKKGLTDEEIDMAFQQSGTAADEPSSLW